European Patent Application EP 4 471 148 A1, published December 4, 2024. Title: PROMOTER, THREONINE-PRODUCING RECOMBINANT MICROORGANISM AND USE THEREOF. Applicant: Langfang Meihua Biotechnology Development Co.,Ltd. Application EP 22923633.6, filed December 28, 2022. The sequence listing filed with the application follows.

SEQUENCE LISTING (39 sequences)

SEQ ID NO: 1 - DNA, 222 bp, synthetic construct
  source 1..222: mol_type = other DNA
tcacacccaagagctaaaaattcatatagttaagacaacattttggctgtaaaagacagccgtaaaaacctcttgctcgtgtcaattgttcttatcggaatgtggcttgggcgattgttatgcaaaagttgttaggttttttgcggggttgtttaacccccaaatgagggaagaaggtagaattgaactctatgagcacaggtttaacagctaagaccggag

SEQ ID NO: 2 - DNA, 46 bp, synthetic construct
  source 1..46: mol_type = other DNA
aattcgagctcggtacccggggatccagcgacaggacaagcactgg

SEQ ID NO: 3 - DNA, 40 bp, synthetic construct
  source 1..40: mol_type = other DNA
cccggaataattggcagctatgtgcacctttcgatctacg

SEQ ID NO: 4 - DNA, 40 bp, synthetic construct
  source 1..40: mol_type = other DNA
cgtagatcgaaaggtgcacatagctgccaattattccggg

SEQ ID NO: 5 - DNA, 41 bp, synthetic construct
  source 1..41: mol_type = other DNA
tttctgtacgaccagggccatgggtaaaaaatcctttcgta

SEQ ID NO: 6 - DNA, 41 bp, synthetic construct
  source 1..41: mol_type = other DNA
tacgaaaggattttttacccatggccctggtcgtacagaaa

SEQ ID NO: 7 - DNA, 42 bp, synthetic construct
  source 1..42: mol_type = other DNA
tcggaacgagggcaggtgaaggtgatgtcggtggtgccgtct

SEQ ID NO: 8 - DNA, 42 bp, synthetic construct
  source 1..42: mol_type = other DNA
agacggcaccaccgacatcaccttcacctgccctcgttccga

SEQ ID NO: 9 - DNA, 46 bp, synthetic construct
  source 1..46: mol_type = other DNA
gtaaaacgacggccagtgccaagcttagcctggtaagaggaaacgt

SEQ ID NO: 10 - DNA, 46 bp, synthetic construct
  source 1..46: mol_type = other DNA
aattcgagctcggtacccggggatccctgcgggcagatccttttga

SEQ ID NO: 11 - DNA, 40 bp, synthetic construct
  source 1..40: mol_type = other DNA
atttctttataaacgcaggtcatatctaccaaaactacgc

SEQ ID NO: 12 - DNA, 40 bp, synthetic construct
  source 1..40: mol_type = other DNA
gcgtagttttggtagatatgacctgcgtttataaagaaat

SEQ ID NO: 13 - DNA, 40 bp, synthetic construct
  source 1..40: mol_type = other DNA
gtatatctccttctgcaggaataggtatcgaaagacgaaa

SEQ ID NO: 14 - DNA, 40 bp, synthetic construct
  source 1..40: mol_type = other DNA
tttcgtctttcgatacctattcctgcagaaggagatatac

SEQ ID NO: 15 - DNA, 41 bp, synthetic construct
  source 1..41: mol_type = other DNA
tagccaattcagccaaaacccccacgcgatcttccacatcc

SEQ ID NO: 16 - DNA, 41 bp, synthetic construct
  source 1..41: mol_type = other DNA
ggatgtggaagatcgcgtgggggttttggctgaattggcta

SEQ ID NO: 17 - DNA, 46 bp, synthetic construct
  source 1..46: mol_type = other DNA
gtaaaacgacggccagtgccaagcttgctggctcttgccgtcgata

SEQ ID NO: 18 - DNA, 56 bp, synthetic construct
  source 1..56: mol_type = other DNA
catgattacgaattcgagctcggtacccggggatcctccgcgacccatgaattggt

SEQ ID NO: 19 - DNA, 50 bp, synthetic construct
  source 1..50: mol_type = other DNA
actatatgaatttttagctcttgggtgtgagctttgcgttaaaagtccat

SEQ ID NO: 20 - DNA, 51 bp, synthetic construct
  source 1..51: mol_type = other DNA
tgagcacaggtttaacagctaagaccggagtagagcacttcggcaccgttg

SEQ ID NO: 21 - DNA, 56 bp, synthetic construct
  source 1..56: mol_type = other DNA
tcacgacgttgtaaaacgacggccagtgccaagcttacccttggcgtccttgaccg

SEQ ID NO: 22 - DNA, 56 bp, synthetic construct
  source 1..56: mol_type = other DNA
catgattacgaattcgagctcggtacccggggatccgtatcggcagttccagccat

SEQ ID NO: 23 - DNA, 50 bp, synthetic construct
  source 1..50: mol_type = other DNA
actatatgaatttttagctcttgggtgtgaatgatgattcagggacatct

SEQ ID NO: 24 - DNA, 51 bp, synthetic construct
  source 1..51: mol_type = other DNA
tgagcacaggtttaacagctaagaccggaggattacaagaacatgaccaac

SEQ ID NO: 25 - DNA, 56 bp, synthetic construct
  source 1..56: mol_type = other DNA
tcacgacgttgtaaaacgacggccagtgccaagctttgaacgccagggatgcgtcg

SEQ ID NO: 26 - DNA, 56 bp, synthetic construct
  source 1..56: mol_type = other DNA
catgattacgaattcgagctcggtacccggggatccacgttgatgccaaactgggt

SEQ ID NO: 27 - DNA, 50 bp, synthetic construct
  source 1..50: mol_type = other DNA
actatatgaatttttagctcttgggtgtgattgtctttgcgtcgaagtac

SEQ ID NO: 28 - DNA, 50 bp, synthetic construct
  source 1..50: mol_type = other DNA
tgagcacaggtttaacagctaagaccggagcactagtcaaccatgagtga

SEQ ID NO: 29 - DNA, 56 bp, synthetic construct
  source 1..56: mol_type = other DNA
tcacgacgttgtaaaacgacggccagtgccaagcttgttgcgccggtgcgctctgc

SEQ ID NO: 30 - DNA, 56 bp, synthetic construct
  source 1..56: mol_type = other DNA
catgattacgaattcgagctcggtacccggggatcccttccatcttctagtggttc

SEQ ID NO: 31 - DNA, 49 bp, synthetic construct
  source 1..49: mol_type = other DNA
actatatgaatttttagctcttgggtgtgaatgcctgcaattgaacttc

SEQ ID NO: 32 - DNA, 50 bp, synthetic construct
  source 1..50: mol_type = other DNA
tgagcacaggtttaacagctaagaccggaggaaaacacaggcatgctcac

SEQ ID NO: 33 - DNA, 56 bp, synthetic construct
  source 1..56: mol_type = other DNA
tcacgacgttgtaaaacgacggccagtgccaagcttacaatttctagcccaatgac

SEQ ID NO: 34 - DNA, 55 bp, synthetic construct
  source 1..55: mol_type = other DNA
catgattacgaattcgagctcggtacccggggatcctttgcgaacttggaggaga

SEQ ID NO: 35 - DNA, 50 bp, synthetic construct
  source 1..50: mol_type = other DNA
actatatgaatttttagctcttgggtgtgagcgttttcaatagttcggtg

SEQ ID NO: 36 - DNA, 51 bp, synthetic construct
  source 1..51: mol_type = other DNA
tgagcacaggtttaacagctaagaccggagccgaacaaatatgtttgaaag

SEQ ID NO: 37 - DNA, 56 bp, synthetic construct
  source 1..56: mol_type = other DNA
tcacgacgttgtaaaacgacggccagtgccaagcttcctcatcgagtgggttcagc

SEQ ID NO: 38 - DNA, 30 bp, synthetic construct
  source 1..30: mol_type = other DNA
tcacacccaagagctaaaaattcatatagt

SEQ ID NO: 39 - DNA, 30 bp, synthetic construct
  source 1..30: mol_type = other DNA
ctccggtcttagctgttaaacctgtgctca